European Patent Application EP 4 253 569 A2, published October 4, 2023. Title: Escherichia Coli-Based Recombinant Strain, Construction Method Therefor and Use Thereof. Applicant: Heilongjiang Eppen Biotech Co Ltd. The sequence listing filed with the application follows.

SEQUENCE LISTING (32 sequences)

SEQ ID NO: 1 - DNA, 1278 bp, Escherichia coli
  source 1..1278: mol_type = genomic DNA
atgctcgaattgctttacaccgcccttctctaccttattcagccgctgatctggatacggctctgggtgcgcggacgtaaggctccggcctatcgaaaacgctggggtgaacgttacggtttttaccgccatccgctaaaaccaggcggcattatgctgcactccgtctccgtcggtgaaactctggcggcaatcccgttggtgcgcgcgctgcgtcatcgttatcctgatttaccgattaccgtaacaaccatgacgccaaccggttcggagcgcgtacaatcggctttcgggaaggatgttcagcacgtttatctgccgtatgatctgcccgatgcactcaaccgtttcctgaataaagtcgaccctaaactggtgttgattatggaaaccgaactatggcctaacctgattgcggcgctacataaacgtaaaattccgctggtgatcgctaacgcgcgactctctgcccgctcggccgcaggttatgccaaactgggtaaattcgtccgtcgcttgctgcgtcgtattacgctgattgctgcgcaaaatgaagaagatggtgcacgttttgtggcgctgggcgcaaaaaataatcaggtgaccgttaccggtagcctgaaattcgatatttctgtaacgccgcagttggctgctaaagccgtgacgctgcgccgccagtgggcaccacaccgcccggtatggattgccaccagcactcacgaaggcgaagagagtgtggtgatcgccgcacatcaggcattgttacagcaattcccgaatttattgctcatcctggtaccccgtcatccggaacgcttcccggatgcgattaaccttgtccgccaggctggactaagctatatcacacgctcttcaggggaagtcccctccaccagcacgcaggttgtggttggcgatacgatgggcgagttgatgttactgtatggcattgccgatctcgcctttgttggcggttcactggttgaacgtggtgggcataatccgctggaagctgccgcacacgctattccggtattgatggggccgcatacttttaactttaaagacatttgcgcgcggctggagcaggcaagcgggctgattaccgttaccgatgccactacgcttgcaaaagaggtttcctctttactcaccgacgccgattaccgtagtttctatggccgtcatgccgttgaagtactgtatcaaaaccagggcgcgctacagcgtctgcttcaactgctggaaccttacctgccaccgaaaacgcattga

SEQ ID NO: 2 - DNA, 1278 bp, synthetic construct
  source 1..1278: mol_type = other DNA
atgctcgaattgctttacaccgcccttctctaccttattcagccgctgatctggatacggctctgggtgcgcggacgtaagactccggcctatcgaaaacgctggggtgaacgttacggtttttaccgccatccgctaaaaccaggcggcattatgctgcactccgtctccgtcggtgaaactctggcggcaatcccgttggtgcgcgcgctgcgtcatcgttatcctgatttaccgattaccgtaacaaccatgacgccaaccggttcggagcgcgtacaatcggctttcgggaaggatgttcagcacgtttatctgccgtatgatctgcccgatgcactcaaccgtttcctgaataaagtcgaccctaaactggtgttgattatggaaaccgaactatggcctaacctgattgcggcgctacataaacgtaaaattccgctggtgatcgctaacgcgcgactctctgcccgctcggccgcaggttatgccaaactgggtaaattcgtccgtcgcttgctgcgtcgtattacgctgattgctgcgcaaaatgaagaagatggtgcacgttttgtggcgctgggcgcaaaaaataatcaggtgaccgttaccggtagcctgaaattcgatatttctgtaacgccgcagttggctgctaaagccgtgacgctgcgccgccagtgggcaccacaccgcccggtatggattgccaccagcactcacgaaggcgaagagagtgtggtgatcgccgcacatcaggcattgttacagcaattcccgaatttattgctcatcctggtaccccgtcatccggaacgcttcccggatgcgattaaccttgtccgccaggctggactaagctatatcacacgctcttcaggggaagtcccctccaccagcacgcaggttgtggttggcgatacgatgggcgagttgatgttactgtatggcattgccgatctcgcctttgttggcggttcactggttgaacgtggtgggcataatccgctggaagctgccgcacacgctattccggtattgatggggccgcatacttttaactttaaagacatttgcgcgcggctggagcaggcaagcgggctgattaccgttaccgatgccactacgcttgcaaaagaggtttcctctttactcaccgacgccgattaccgtagtttctatggccgtcatgccgttgaagtactgtatcaaaaccagggcgcgctacagcgtctgcttcaactgctggaaccttacctgccaccgaaaacgcattga

SEQ ID NO: 3 - protein, 425 aa, Escherichia coli
MLELLYTALLYLIQPLIWIRLWVRGRKAPAYRKRWGERYGFYRHPLKPGGIMLHSVSVGETLAAIPLVRALRHRYPDLPITVTTMTPTGSERVQSAFGKDVQHVYLPYDLPDALNRFLNKVDPKLVLIMETELWPNLIAALHKRKIPLVIANARLSARSAAGYAKLGKFVRRLLRRITLIAAQNEEDGARFVALGAKNNQVTVTGSLKFDISVTPQLAAKAVTLRRQWAPHRPVWIATSTHEGEESVVIAAHQALLQQFPNLLLILVPRHPERFPDAINLVRQAGLSYITRSSGEVPSTSTQVVVGDTMGELMLLYGIADLAFVGGSLVERGGHNPLEAAAHAIPVLMGPHTFNFKDICARLEQASGLITVTDATTLAKEVSSLLTDADYRSFYGRHAVEVLYQNQGALQRLLQLLEPYLPPKTH

SEQ ID NO: 4 - protein, 425 aa, synthetic construct
MLELLYTALLYLIQPLIWIRLWVRGRKTPAYRKRWGERYGFYRHPLKPGGIMLHSVSVGETLAAIPLVRALRHRYPDLPITVTTMTPTGSERVQSAFGKDVQHVYLPYDLPDALNRFLNKVDPKLVLIMETELWPNLIAALHKRKIPLVIANARLSARSAAGYAKLGKFVRRLLRRITLIAAQNEEDGARFVALGAKNNQVTVTGSLKFDISVTPQLAAKAVTLRRQWAPHRPVWIATSTHEGEESVVIAAHQALLQQFPNLLLILVPRHPERFPDAINLVRQAGLSYITRSSGEVPSTSTQVVVGDTMGELMLLYGIADLAFVGGSLVERGGHNPLEAAAHAIPVLMGPHTFNFKDICARLEQASGLITVTDATTLAKEVSSLLTDADYRSFYGRHAVEVLYQNQGALQRLLQLLEPYLPPKTH

SEQ ID NO: 5 - DNA, 26 bp, synthetic construct
  source 1..26: mol_type = other DNA
cgggatccaccagtgaaccgccaaca

SEQ ID NO: 6 - DNA, 18 bp, synthetic construct
  source 1..18: mol_type = other DNA
tgcgcggacgtaagactc

SEQ ID NO: 7 - DNA, 18 bp, synthetic construct
  source 1..18: mol_type = other DNA
gagtcttacgtccgcgca

SEQ ID NO: 8 - DNA, 35 bp, synthetic construct
  source 1..35: mol_type = other DNA
aaggaaaaaagcggccgcttcccgcacctttattg

SEQ ID NO: 9 - DNA, 18 bp, synthetic construct
  source 1..18: mol_type = other DNA
cttcccgaaagccgattg

SEQ ID NO: 10 - DNA, 18 bp, synthetic construct
  source 1..18: mol_type = other DNA
acaaaatatactttaatc

SEQ ID NO: 11 - DNA, 1596 bp, synthetic construct
  source 1..1596: mol_type = other DNA
accagtgaaccgccaacaaaggcgagatcggcaatgccatacagtaacatcaactcgcccatcgtatcgccaaccacaacctgcgtgctggtggaggggacttcccctgaagagcgtgtgatatagcttagtccagcctggcggacaaggttaatcgcatccgggaagcgttccggatgacggggtaccaggatgagcaataaattcgggaattgctgtaacaatgcctgatgtgcggcgatcaccacactctcttcgccttcgtgagtgctggtggcaatccataccgggcggtgtggtgcccactggcggcgcagcgtcacggctttagcagccaactgcggcgttacagaaatatcgaatttcaggctaccggtaacggtcacctgattattttttgcgcccagcgccacaaaacgtgcaccatcttcttcattttgcgcagcaatcagcgtaatacgacgcagcaagcgacggacgaatttacccagtttggcataacctgcggccgagcgggcagagagtcgcgcgttagcgatcaccagcggaattttacgtttatgtagcgccgcaatcaggttaggccatagttcggtttccataatcaacaccagtttagggtcgactttattcaggaaacggttgagtgcatcgggcagatcatacggcagataaacgtgctgaacatccttcccgaaagccgattgtacgcgctccgaaccggttggcgtcatggttgttacggtaatcggtaaatcaggataacgatgacgcagcgcgcgcaccaacgggattgccgccagagtttcaccgacggagacggagtgcagcataatgccgcctggttttagcggatggcggtaaaaaccgtaacgttcaccccagcgttttcgataggccggagacttacgtccgcgcacccagagccgtatccagatcagcggctgaataaggtagagaagggcggtgtaaagcaattcgagcatagtaaatagctgacttatggatgtgctggggattctatgtatttagctgtggctttaccattacttttcccgtttttgacttaaatagcttcagtttggtctgatctgccgctacatcttcattttttttgtatttttatgcgattcattgaaactcggccccattttcaaatctacataggccgtactgacattatcgaaatgctattttttatctatttgatttttatgattaaagtatattttgtgtataaaaatcattcgggtcggattgctgcgaaagaaatgatacactagcacgtcaaagtaagtgcgttatcagtattcaggtagctgttgagcctggggcggtagcgtgcttttttctgcttaacttaaccagacaatcacacaaaagagtcgctagtggaaaagccatttcgaaaaatcctggtcataaagatgcgatatcatggggatatgttattaactactcctgtcatcagtacgctcaagcagaattatcctgatgcaaaaatcgatatgctgctttatcaggacaccatccctattttgtctgaaaacccggaaattaatgcgctctatgggataagcaataaaggtgcgggaa

SEQ ID NO: 12 - DNA, 544 bp, synthetic construct
  source 1..544: mol_type = other DNA
cttcccgaaagccgattgtacgcgctccgaaccggttggcgtcatggttgttacggtaatcggtaaatcaggataacgatgacgcagcgcgcgcaccaacgggattgccgccagagtttcaccgacggagacggagtgcagcataatgccgcctggttttagcggatggcggtaaaaaccgtaacgttcaccccagcgttttcgataggccggagacttacgtccgcgcacccagagccgtatccagatcagcggctgaataaggtagagaagggcggtgtaaagcaattcgagcatagtaaatagctgacttatggatgtgctggggattctatgtatttagctgtggctttaccattacttttcccgtttttgacttaaatagcttcagtttggtctgatctgccgctacatcttcattttttttgtatttttatgcgattcattgaaactcggccccattttcaaatctacataggccgtactgacattatcgaaatgctattttttatctatttgatttttatgattaaagtatattttg

SEQ ID NO: 13 - DNA, 2109 bp, Escherichia coli
  source 1..2109: mol_type = genomic DNA
atgtatctgtttgaaagcctgaatcaactgattcaaacctacctgccggaagaccaaatcaagcgtctgcggcaggcgtatctcgttgcacgtgatgctcacgaggggcaaacacgttcaagcggtgaaccctatatcacgcacccggtagcggttgcctgcattctggccgagatgaaactcgactatgaaacgctgatggcggcgctgctgcatgacgtgattgaagatactcccgccacctaccaggatatggaacagctttttggtaaaagcgtcgccgagctggtagagggggtgtcgaaacttgataaactcaagttccgcgataagaaagaggcgcaggccgaaaactttcgcaagatgattatggcgatggtgcaggatatccgcgtcatcctcatcaaacttgccgaccgtacccacaacatgcgcacgctgggctcacttcgcccggacaaacgtcgccgcatcgcccgtgaaactctcgaaatttatagcccgctggcgcaccgtttaggtatccaccacattaaaaccgaactcgaagagctgggttttgaggcgctgtatcccaaccgttatcgcgtaatcaaagaagtggtgaaagccgcgcgcggcaaccgtaaagagatgatccagaagattctttctgaaatcgaagggcgtttgcaggaagcgggaataccgtgccgcgtcagtggtcgcgagaagcatctttattcgatttactgcaaaatggtgctcaaagagcagcgttttcactcgatcatggacatctacgctttccgcgtgatcgtcaatgattctgacacctgttatcgcgtgctgggccagatgcacagcctgtacaagccgcgtccgggccgcgtgaaagactatatcgccattccaaaagcgaacggctatcagtctttgcacacctcgatgatcggcccgcacggtgtgccggttgaggtccagatccgtaccgaagatatggaccagatggcggagatgggtgttgccgcgcactgggcttataaagagcacggcgaaaccagtactaccgcacaaatccgcgcccagcgctggatgcaaagcctgctggagctgcaacagagcgccggtagttcgtttgaatttatcgagagcgttaaatccgatctcttcccggatgagatttacgttttcacaccggaagggcgcattgtcgagctgcctgccggtgcaacgcccgtcgacttcgcttatgcagtgcataccgatatcggtcatgcctgcgtgggcgcacgcgttgaccgccagccttacccgctgtcgcagccgcttaccagcggtcaaaccgttgaaatcattaccgctccgggcgctcgcccgaatgccgcttggctgaactttgtcgttagctcgaaagcgcgcgccaaaattcgtcagttgctgaaaaacctcaagcgtgatgattctgtaagcctgggccgtcgtctgctcaaccatgctttgggtggtagccgtaagctgaatgaaatcccgcaggaaaatattcagcgcgagctggatcgcatgaagctggcaacgcttgacgatctgctggcagaaatcggacttggtaacgcaatgagcgtggtggtcgcgaaaaatctgcaacatggggacgcctccattccaccggcaacccaaagccacggacatctgcccattaaaggtgccgatggcgtgctgatcacctttgcgaaatgctgccgccctattcctggcgacccgattatcgcccacgtcagccccggtaaaggtctggtgatccaccatgaatcctgccgtaatatccgtggctaccagaaagagccagagaagtttatggctgtggaatgggataaagagacggcgcaggagttcatcaccgaaatcaaggtggagatgttcaatcatcagggtgcgctggcaaacctgacggcggcaattaacaccacgacttcgaatattcaaagtttgaatacggaagagaaagatggtcgcgtctacagcgcctttattcgtctgaccgctcgtgaccgtgtgcatctggcgaatatcatgcgcaaaatccgcgtgatgccagacgtgattaaagtcacccgaaaccgaaattaa

SEQ ID NO: 14 - DNA, 2109 bp, synthetic construct
  source 1..2109: mol_type = other DNA
atgtatctgtttgaaagcctgaatcaactgattcaaacctacctgccggaagaccaaatcaagcgtctgcggcaggcgtatctcgttgcacgtgatgctcacgaggggcaaacacgttcaagcggtgaaccctatatcacgcacccggtagcggttgcctgcattctggccgagatgaaactcgactatgaaacgctgatggcggcgctgctgcatgacgtgattgaagatactcccgccacctaccaggatatggaacagctttttggtaaaagcgtcgccgagctggtagagggggtgtcgaaacttgataaactcaagttccgcgataagaaagaggcgcaggccgaaaactttcgcaagatgattatggcgatggtgcaggatatccgcgtcatcctcatcaaacttgccgaccgtacccacaacatgcgcacgctgggctcacttcgcccggacaaacgtcgccgcatcgcccgtgaaactctcgaaatttatagcccgctggcgcaccgtttatgtatccaccacattaaaaccgaactcgaagagctgggttttgaggcgctgtatcccaaccgttatcgcgtaatcaaagaagtggtgaaagccgcgcgcggcaaccgtaaagagatgatccagaagattctttctgaaatcgaagggcgtttgcaggaagcgggaataccgtgccgcgtcagtggtcgcgagaagcatctttattcgatttactgcaaaatggtgctcaaagagcagcgttttcactcgatcatggacatctacgctttccgcgtgatcgtcaatgattctgacacctgttatcgcgtgctgggccagatgcacagcctgtacaagccgcgtccgggccgcgtgaaagactatatcgccattccaaaagcgaacggctatcagtctttgcacacctcgatgatcggcccgcacggtgtgccggttgaggtccagatccgtaccgaagatatggaccagatggcggagatgggtgttgccgcgcactgggcttataaagagcacggcgaaaccagtactaccgcacaaatccgcgcccagcgctggatgcaaagcctgctggagctgcaacagagcgccggtagttcgtttgaatttatcgagagcgttaaatccgatctcttcccggatgagatttacgttttcacaccggaagggcgcattgtcgagctgcctgccggtgcaacgcccgtcgacttcgcttatgcagtgcataccgatatcggtcatgcctgcgtgggcgcacgcgttgaccgccagccttacccgctgtcgcagccgcttaccagcggtcaaaccgttgaaatcattaccgctccgggcgctcgcccgaatgccgcttggctgaactttgtcgttagctcgaaagcgcgcgccaaaattcgtcagttgctgaaaaacctcaagcgtgatgattctgtaagcctgggccgtcgtctgctcaaccatgctttgggtggtagccgtaagctgaatgaaatcccgcaggaaaatattcagcgcgagctggatcgcatgaagctggcaacgcttgacgatctgctggcagaaatcggacttggtaacgcaatgagcgtggtggtcgcgaaaaatctgcaacatggggacgcctccattccaccggcaacccaaagccacggacatctgcccattaaaggtgccgatggcgtgctgatcacctttgcgaaatgctgccgccctattcctggcgacccgattatcgcccacgtcagccccggtaaaggtctggtgatccaccatgaatcctgccgtaatatccgtggctaccagaaagagccagagaagtttatggctgtggaatgggataaagagacggcgcaggagttcatcaccgaaatcaaggtggagatgttcaatcatcagggtgcgctggcaaacctgacggcggcaattaacaccacgacttcgaatattcaaagtttgaatacggaagagaaagatggtcgcgtctacagcgcctttattcgtctgaccgctcgtgaccgtgtgcatctggcgaatatcatgcgcaaaatccgcgtgatgccagacgtgattaaagtcacccgaaaccgaaattaa

SEQ ID NO: 15 - protein, 702 aa, Escherichia coli
MYLFESLNQLIQTYLPEDQIKRLRQAYLVARDAHEGQTRSSGEPYITHPVAVACILAEMKLDYETLMAALLHDVIEDTPATYQDMEQLFGKSVAELVEGVSKLDKLKFRDKKEAQAENFRKMIMAMVQDIRVILIKLADRTHNMRTLGSLRPDKRRRIARETLEIYSPLAHRLGIHHIKTELEELGFEALYPNRYRVIKEVVKAARGNRKEMIQKILSEIEGRLQEAGIPCRVSGREKHLYSIYCKMVLKEQRFHSIMDIYAFRVIVNDSDTCYRVLGQMHSLYKPRPGRVKDYIAIPKANGYQSLHTSMIGPHGVPVEVQIRTEDMDQMAEMGVAAHWAYKEHGETSTTAQIRAQRWMQSLLELQQSAGSSFEFIESVKSDLFPDEIYVFTPEGRIVELPAGATPVDFAYAVHTDIGHACVGARVDRQPYPLSQPLTSGQTVEIITAPGARPNAAWLNFVVSSKARAKIRQLLKNLKRDDSVSLGRRLLNHALGGSRKLNEIPQENIQRELDRMKLATLDDLLAEIGLGNAMSVVVAKNLQHGDASIPPATQSHGHLPIKGADGVLITFAKCCRPIPGDPIIAHVSPGKGLVIHHESCRNIRGYQKEPEKFMAVEWDKETAQEFITEIKVEMFNHQGALANLTAAINTTTSNIQSLNTEEKDGRVYSAFIRLTARDRVHLANIMRKIRVMPDVIKVTRNRN

SEQ ID NO: 16 - protein, 702 aa, synthetic construct
MYLFESLNQLIQTYLPEDQIKRLRQAYLVARDAHEGQTRSSGEPYITHPVAVACILAEMKLDYETLMAALLHDVIEDTPATYQDMEQLFGKSVAELVEGVSKLDKLKFRDKKEAQAENFRKMIMAMVQDIRVILIKLADRTHNMRTLGSLRPDKRRRIARETLEIYSPLAHRLCIHHIKTELEELGFEALYPNRYRVIKEVVKAARGNRKEMIQKILSEIEGRLQEAGIPCRVSGREKHLYSIYCKMVLKEQRFHSIMDIYAFRVIVNDSDTCYRVLGQMHSLYKPRPGRVKDYIAIPKANGYQSLHTSMIGPHGVPVEVQIRTEDMDQMAEMGVAAHWAYKEHGETSTTAQIRAQRWMQSLLELQQSAGSSFEFIESVKSDLFPDEIYVFTPEGRIVELPAGATPVDFAYAVHTDIGHACVGARVDRQPYPLSQPLTSGQTVEIITAPGARPNAAWLNFVVSSKARAKIRQLLKNLKRDDSVSLGRRLLNHALGGSRKLNEIPQENIQRELDRMKLATLDDLLAEIGLGNAMSVVVAKNLQHGDASIPPATQSHGHLPIKGADGVLITFAKCCRPIPGDPIIAHVSPGKGLVIHHESCRNIRGYQKEPEKFMAVEWDKETAQEFITEIKVEMFNHQGALANLTAAINTTTSNIQSLNTEEKDGRVYSAFIRLTARDRVHLANIMRKIRVMPDVIKVTRNRN

SEQ ID NO: 17 - DNA, 28 bp, synthetic construct
  source 1..28: mol_type = other DNA
cgggatccgaacagcaagagcaggaagc

SEQ ID NO: 18 - DNA, 19 bp, synthetic construct
  source 1..19: mol_type = other DNA
tgtggtggatacataaacg

SEQ ID NO: 19 - DNA, 20 bp, synthetic construct
  source 1..20: mol_type = other DNA
gcaccgtttatgtatccacc

SEQ ID NO: 20 - DNA, 38 bp, synthetic construct
  source 1..38: mol_type = other DNA
aaggaaaaaagcggccgcacgacaaagttcagccaagc

SEQ ID NO: 21 - DNA, 20 bp, synthetic construct
  source 1..20: mol_type = other DNA
ctttcgcaagatgattatgg

SEQ ID NO: 22 - DNA, 20 bp, synthetic construct
  source 1..20: mol_type = other DNA
cacggtattcccgcttcctg

SEQ ID NO: 23 - DNA, 567 bp, Escherichia coli
  source 1..567: mol_type = genomic DNA
atgaatatcactgctactgttcttcttgcgtttggtatgtcgatggatgcatttgctgcatcaatcggtaaaggtgccaccctccataaaccgaaattttctgaagcattgcgaaccggccttatttttggtgccgtcgaaaccctgacgccgctgatcggctggggaatgggcatgttagccagccggtttgtccttgaatggaaccactggattgcgtttgtgctgctgatattcctcggcgggcgaatgattattgagggttttcgtggcgcagatgatgaagatgaagagccgcgccgtcgacacggtttctggctactggtaaccaccgcgattgccaccagcctggatgccatggctgtgggtgttggtcttgctttcctgcaggtcaacattatcgcgaccgcattggccattggttgtgcaaccttgattatgtcaacattagggatgatggttggtcgctttatcggctcaattattgggaaaaaagcggaaattctcggcgggctggtgctgatcggcatcggcgtccagatcctctggacgcacttccacggttaa

SEQ ID NO: 24 - DNA, 567 bp, synthetic construct
  source 1..567: mol_type = other DNA
atgaatatcactgctactgttcttcttgcgtttggtatgtcgatggatgcatttgctgcatcaatcggtaaagatgccaccctccataaaccgaaattttctgaagcattgcgaaccggccttatttttggtgccgtcgaaaccctgacgccgctgatcggctggggaatgggcatgttagccagccggtttgtccttgaatggaaccactggattgcgtttgtgctgctgatattcctcggcgggcgaatgattattgagggttttcgtggcgcagatgatgaagatgaagagccgcgccgtcgacacggtttctggctactggtaaccaccgcgattgccaccagcctggatgccatggctgtgggtgttggtcttgctttcctgcaggtcaacattatcgcgaccgcattggccattggttgtgcaaccttgattatgtcaacattagggatgatggttggtcgctttatcggctcaattattgggaaaaaagcggaaattctcggcgggctggtgctgatcggcatcggcgtccagatcctctggacgcacttccacggttaa

SEQ ID NO: 25 - protein, 188 aa, Escherichia coli
MNITATVLLAFGMSMDAFAASIGKGATLHKPKFSEALRTGLIFGAVETLTPLIGWGMGMLASRFVLEWNHWIAFVLLIFLGGRMIIEGFRGADDEDEEPRRRHGFWLLVTTAIATSLDAMAVGVGLAFLQVNIIATALAIGCATLIMSTLGMMVGRFIGSIIGKKAEILGGLVLIGIGVQILWTHFHG

SEQ ID NO: 26 - protein, 188 aa, synthetic construct
MNITATVLLAFGMSMDAFAASIGKDATLHKPKFSEALRTGLIFGAVETLTPLIGWGMGMLASRFVLEWNHWIAFVLLIFLGGRMIIEGFRGADDEDEEPRRRHGFWLLVTTAIATSLDAMAVGVGLAFLQVNIIATALAIGCATLIMSTLGMMVGRFIGSIIGKKAEILGGLVLIGIGVQILWTHFHG

SEQ ID NO: 27 - DNA, 28 bp, synthetic construct
  source 1..28: mol_type = other DNA
cgggatcccttcgccaatgtctggattg

SEQ ID NO: 28 - DNA, 20 bp, synthetic construct
  source 1..20: mol_type = other DNA
atggagggtggcatctttac

SEQ ID NO: 29 - DNA, 20 bp, synthetic construct
  source 1..20: mol_type = other DNA
tgcatcaatcggtaaagatg

SEQ ID NO: 30 - DNA, 38 bp, synthetic construct
  source 1..38: mol_type = other DNA
aaggaaaaaagcggccgccaactccgcactctgctgta

SEQ ID NO: 31 - DNA, 19 bp, synthetic construct
  source 1..19: mol_type = other DNA
ccatcacggcttgttgttc

SEQ ID NO: 32 - DNA, 19 bp, synthetic construct
  source 1..19: mol_type = other DNA
acgaaaaccctcaataatc